European Patent Application EP 4 589 019 A1, published July 23, 2025. Title: 多重PCR反应体系. Applicant: 迈克生物股份有限公司. Application CN. The sequence listing filed with the application follows.

SEQUENCE LISTING (19 sequences)

SEQ ID NO: 1 - DNA, 59 bp, synthetic construct
  source 1..59: mol_type = other DNA; note = Spacer C3 is added between c15 and t16; t16 is modified with ROX; t28 is modified with BHQ2; c59 is modified with Spacer C3.
aggacgtgacgtctctcagcacgtagctcctcgatgcctgcgctcctgtacctgactgc

SEQ ID NO: 2 - DNA, 34 bp, synthetic construct
  source 1..34: mol_type = other DNA
tcagcacgtagctaaatcgtcgggctggtagttg

SEQ ID NO: 3 - DNA, 35 bp, synthetic construct
  source 1..35: mol_type = other DNA
acgtcacgtcctaaacgatgaagcagatggcgtta

SEQ ID NO: 4 - DNA, 59 bp, synthetic construct
  source 1..59: mol_type = other DNA; note = note = BHQ2 is added between a16 and t17; t30 is modified with FAM; c59 is modified with Spacer C3.
cctctcctacttggcatctcgatgactgatcgcacagtccgtacccgatcggctgacga

SEQ ID NO: 5 - DNA, 33 bp, synthetic construct
  source 1..33: mol_type = other DNA
cggctgacgaaaaacgcacaaccgaagcgtaga

SEQ ID NO: 6 - DNA, 37 bp, synthetic construct
  source 1..37: mol_type = other DNA
gccaagtaggagaggaaagaaccggacagagcccatt

SEQ ID NO: 7 - DNA, 33 bp, synthetic construct
  source 1..33: mol_type = other DNA
acgtcacgtcctaaaaggagcgacccagaaagt

SEQ ID NO: 8 - DNA, 33 bp, synthetic construct
  source 1..33: mol_type = other DNA
acctgactgcaaagctctgtgcataactgtggt

SEQ ID NO: 9 - DNA, 38 bp, synthetic construct
  source 1..38: mol_type = other DNA
acgtcacgtcctaaatggatcagccattgtagttacag

SEQ ID NO: 10 - DNA, 31 bp, synthetic construct
  source 1..31: mol_type = other DNA
gcgctcctgtaaatggaatcgtgtgccccaa

SEQ ID NO: 11 - DNA, 37 bp, synthetic construct
  source 1..37: mol_type = other DNA
acgtcacgtcctaaacgcctcacatttacaacaggac

SEQ ID NO: 12 - DNA, 34 bp, synthetic construct
  source 1..34: mol_type = other DNA
ctcgatgcctaaaacaagcaaaaccagacacctc

SEQ ID NO: 13 - DNA, 59 bp, synthetic construct
  source 1..59: mol_type = other DNA; note = t31 is modified with CY5; t47 is modified with BHQ2; Spacer C3 is added between g39 and c40; c59 is modified with Spacer C3.
cctgcgacgctcatctcagtacagcgtctgtcgctgatgcgcacactgggaccaccgct

SEQ ID NO: 14 - DNA, 34 bp, synthetic construct
  source 1..34: mol_type = other DNA
gaccaccgctaaaagtctgaacgacctacactcc

SEQ ID NO: 15 - DNA, 34 bp, synthetic construct
  source 1..34: mol_type = other DNA
gtcgctgatgaaaagtctgaacgacctacactcc

SEQ ID NO: 16 - DNA, 34 bp, synthetic construct
  source 1..34: mol_type = other DNA
gatgagcgtcgcaggtttcccagcagctgacaca

SEQ ID NO: 17 - DNA, 59 bp, synthetic construct; identical to SEQ ID NO: 1
  source 1..59: mol_type = other DNA; note = t16 is modified with ROX; t28 is modified with BHQ2; c59 is modified with spacer C3.

SEQ ID NO: 18 - DNA, 33 bp, synthetic construct
  source 1..33: mol_type = other DNA
acgtcacgtcctaaaaagggcaacggcatggca

SEQ ID NO: 19 - DNA, 36 bp, synthetic construct
  source 1..36: mol_type = other DNA
acctgactgcaaagcagtttgtatggtcgttgtgta